European Patent Specification EP 3 568 133 B1, published December 13, 2023. Title: CELL-PROTECTIVE COMPOUNDS AND THEIR USE. Applicant: ETH Zurich. The sequence listing filed with the application follows.

SEQUENCE LISTING (10 sequences)

SEQ ID NO: 1 - DNA, 64 bp, Artificial Sequence
  miSrsf top strand
tgctgtttaagtcctgccagcttccagttttggccactgactgactggaagctcaggacttaaa

SEQ ID NO: 2 - DNA, 64 bp, Artificial Sequence
  miSrsf1 bottom strand
cctgtttaagtcctgagcttccagtcagtcagtggccaaaactggaagctggcaggacttaaac

SEQ ID NO: 3 - DNA, 21 bp, Artificial Sequence
  Camk2d-forward primer
acgagaaatttttcagcagcc

SEQ ID NO: 4 - DNA, 21 bp, Artificial Sequence
  Camk2d-reverse-A primer
acagtagtttggggctccagc

SEQ ID NO: 5 - DNA, 21 bp, Artificial Sequence
  Camk2d-reverse-B primer
tcatctgaacactcgaactgg

SEQ ID NO: 6 - DNA, 21 bp, Artificial Sequence
  Camk2d-reverse-C primer
ctcagttgactcctttacccc

SEQ ID NO: 7 - protein, 248 aa, Homo sapiens
MSGGGVIRGPAGNNDCRIYVGNLPPDIRTKDIEDVFYKYGAIRDIDLKNRRGGPPFAFVEFEDPRDAEDAVYGRDGYDYDGYRLRVEFPRSGRGTGRGGGGGGGGGAPRGRYGPPSRRSENRVVVSGLPPSGSWQDLKDHMREAGDVCYADVYRDGTGVVEFVRKEDMTYAVRKLDNTKFRSHEGETAYIRVKVDGPRSPSYGRSRSRSRSRSRSRSRSNSRSRSYSPRRSRGSPRYSPRHSRSRSRT

SEQ ID NO: 8 - protein, 15 aa, Artificial Sequence
  phospho-containing peptide of SRSF1 identfied in Nano-LC-ESI-MS/MS analysis
  MOD_RES (9)..(9): PHOSPHORYLATION
  MOD_RES (11)..(11): PHOSPHORYLATION
RVKVDGPRSPSYGRS

SEQ ID NO: 9 - protein, 13 aa, Artificial Sequence
  phospho-containing peptide of SRSF1 identfied in Nano-LC-ESI-MS/MS analysis
  MOD_RES (7)..(7): PHOSPHORYLATION
  MOD_RES (9)..(9): PHOSPHORYLATION
KVDGPRSPSYGRS

SEQ ID NO: 10 - protein, 236 aa, Artificial Sequence
  carboxyl terminal domain of human GRK2, amino acids 454-689
RSLDWQMVFLQKYPPPLIPPRGEVNAADAFDIGSFDEEDTKGIKLLDSDQELYRNFPLTISERWQQEVAETVFDTINAETDRLEARKKAKNKQLGHEEDYALGKDCIMHGYMSKMGNPFLTQWQRRYFYLFPNRLEWRGEGEAPQSLLTMEEIQSVEETQIKERKCLLLKIRGGKQFILQCDSDPELVQWKKELRDAYREAQQLVQRVPKMKNKPRSPVVELSKVPLVQRGSANGL